European Patent Specification EP 3 502 127 B1, published July 26, 2023. Title: Transgenic Corn Event MON87403 and Methods for Detection Thereof. Applicant: Monsanto Technology LLC. The sequence listing filed with the application follows.

SEQUENCE LISTING (29 sequences)

SEQ ID NO: 1 - DNA, 20 bp, Zea mays
tgatgtttttactgaaggcg

SEQ ID NO: 2 - DNA, 20 bp, Zea mays
tactcattgcgatccacatt

SEQ ID NO: 3 - DNA, 60 bp, Zea mays
tacttaatatgggcacacagtgatgtttttactgaaggcgggaaacgacaatctggcgcg

SEQ ID NO: 4 - DNA, 60 bp, Zea mays
tttctccatattgaccatcatactcattgcgatccacatttccctacatggtggaggata

SEQ ID NO: 5 - DNA, 100 bp, Zea mays
tatgaacccataaaactgaatacttaatatgggcacacagtgatgtttttactgaaggcgggaaacgacaatctggcgcgcctgcctgcaggcatcgttg

SEQ ID NO: 6 - DNA, 100 bp, Zea mays
attggtaattactctttctttttctccatattgaccatcatactcattgcgatccacatttccctacatggtggaggatacagagcactcattccggagt

SEQ ID NO: 7 - DNA, 3000 bp, Zea mays
ctactattttggaacagagggaatagtaggtagtaatgtttcacaataaatcacagtgctaaaatgagatatgaccttagatcccatagctcattgcataaaagtacttgatcagttggtcactgtctttcagaaaaaccgcagtttaattaaacttaatggctgctggatcagatgctagatagcactatatcttaattcgttttgcatgaacaccttataatacagaaccttttcttttcttccagcaactagactctgcatcccttgtggaaatgtgaaccttggttcgtacatgacaaataatacaacatatcatgctacctatgcaacactgacttgatttcaatccttggtttacttgccacatcatacttatggtatatttgggtgaaaagtagatgtttcaagcagtttgtaaatcctaaatacatcatggtttactctggtgctacaactactgttttaaggagaaactattagctttgggatcatctagaatattagcatagcatcaacttcaggcacaactacaagagcagcacttgaaggggtaaaattcagtgctacctacgtaaatcataaaaaaaattatttgtttgaattcaagtgttttgggggttcaacaatgattctatgtagctataaatttttttgttgatttcatgtcatattgattattggtttgatttcacctgttttcttattgtcagccagaaccagcttactatttcggatgttgcaaggaaggcattccttcacagtgtatgtgatagttctctttatacatgtaagacagtgtacaagggcaaaactttgtatgaaattactctgtactgtttacaatgattacagggcatacttgtagtgtttgaggagcaagagacaaaactctacattttagatatataaagcaatagttctttaactcaaaccaaaatctggattagtcttgagcactttctaataatcatataatgctcatgtacctcaataactgcttcagttaatcacatcttttagtttagcactatgctatgatagtttacaaagtgcattgttagcttattttccccataggttctttaatcatatctattgtgctagattttactctgtcccattaggagacaaacaagttcgttcaatagcatatgacacttgtatgctggtaaaatgattgaatattttgtttgacacctattgtttgaaggatgtaagcaatctcatgtacctgttgttgctcgcaaggttcatccctcacaagtacaagatcaaagactcgaaagcttaggtatgaacccataaaactgaatacttaatatgggcacacagtgatgtttttactgaaggcgggaaacgacaatctggcgcgcctgcctgcaggcatcgttgaagatgcctctgccgacagtggtcccaaagatggacccccacccacgaggagcatcgtggaaaaagaagacgttccaaccacgtcttcaaagcaagtggattgatgtgatatctccactgacgtaagggatgacgcacaatcccactatccttcgaggcctcatcgttgaagatgcctctgccgacagtggtcccaaagatggacccccacccacgaggagcatcgtggaaaaagaagacgttccaaccacgtcttcaaagcaagtggattgatgtgatatctccactgacgtaagggatgacgcacaatcccactatccttcgaagcttactcgaggtcattcatatgcttgagaagagagtcgggatagtccaaaataaaacaaaggtaagattacctggtcaaaagtgaaaacatcagttaaaaggtggtataaagtaaaatatcggtaataaaaggtggcccaaagtgaaatttactcttttctactattataaaaattgaggatgtttttgtcggtactttgatacgtcatttttgtatgaattggtttttaagtttattcgcttttggaaatgcatatctgtatttgagtcgggttttaagttcgtttgcttttgtaaatacagagggatttgtataagaaatatctttagaaaaacccatatgctaatttgacataatttttgagaaaaatatatattcaggcgaattctcacaatgaacaataataagattaaaatagctttcccccgttgcagcgcatgggtattttttctagtaaaaataaaagataaacttagactcaaaacatttacaaaaacaacccctaaagttcctaaagcccaaagtgctatccacgatccatagcaagcccagcccaacccaacccaacccaacccaccccagtccagccaactggacaatagtctccacacccccccactatcaccgtgagttgtccgcacgcaccgcacgtctcgcagccaaaaaaaaaaagaaagaaaaaaaagaaaaagaaaaaacagcaggtgggtccgggtcgtgggggccggaaacgcgaggaggatcgcgagccagcgacgaggccggccctccctccgcttccaaagaaacgccccccatcgccactatatacatacccccccctctcctcccatccccccaacccttctagaaccatcttccacacactcaagccacactattggagaacacacagggacaacacaccataagatccaagggaggcctccgccgccgccggtaaccaccccgcccctctcctctttctttctccgtttttttttccgtctcggtctcgatctttggccttggtagtttgggtgggcgagaggcggcttcgtgcgcgcccagatcggtgcgcgggaggggcgggatctcgcggctggggctctcgccggcgtggatccggcccggatctcgcggggaatggggctctcggatgtagatctgcgatccgccgttgttgggggagatgatggggggtttaaaatttccgccgtgctaaacaagatcaggaagaggggaaaagggcactatggtttatatttttatatatttctgctgcttcgtcaggctta

SEQ ID NO: 8 - DNA, 2624 bp, Zea mays
taggtagaagcggaccggtaccatgataaaactactatttacgtacatatgcacatacacatataaactatatgctctatatcatatggattacgcatgcgtgtgtatgtataaatataaaggcatcgtcacgcttcaagtttgtctcttttatattaaactgagagttttcctctcaaactttaccttttcttcttcgatcctagctcttaagaaccctaataattcattgatcaaaataatggcgattttgccggaaaactcttcaaacttggatcttactatctccgttccaggcttctcttcatcccctctctccgatgaaggaagtggcggaggaagagaccagctaaggctagacatgaatcggttaccgtcgtctgaagacggagacgatgaagaattcagtcacgatgatggctctgctcctccgcgaaagaaactccgtctaaccagagaacagtcacgtcttcttgaagatagtttcagacagaatcatacccttaatcccaaacaaaaggaagtacttgccaagcatttgatgctacggccaagacaaattgaagtttggtttcaaaaccgtagagcaaggagcaaattgaagcaaaccgagatggaatgcgagtatctcaaaaggtggtttggttcattaacggaagaaaaccacaggctccatagagaagtagaagagcttagagccataaaggttggcccaacaacggtgaactctgcctcgagccttactatgtgtcctcgctgcgagcgagttacccctgccgcgagcccttcgagggcggtggtgccggttccggctaagaaaacgtttccgccgcaagagcgtgatcgttgagtcggggcccgggctgcatgcgtttggacgtatgctcattcaggttggagccaatttggttgatgtgtgtgcgagttcttgcgagtctgatgagacatctctgtattgtgtttctttccccagtgttttctgtacttgtgtaatcggctaatcgccaacagattcggcgatgaataaatgagaaataaattgttctgattttgagtgcaaaaaaaaaggaattaagcttactcgagatccactagtgattaagcggccgcatcgatcgtgaagtttctcatctaagcccccatttggacgtgaatgtagacacgtcgaaataaagatttccgaattagaataatttgtttattgctttcgcctataaatacgacggatcgtaatttgtcgttttatcaaaatgtactttcattttataataacgctgcggacatctacatttttgaattgaaaaaaaattggtaattactctttctttttctccatattgaccatcatactcattgcgatccacatttccctacatggtggaggatacagagcactcattccggagtataatcttgtcttgtgttgccacctatttatcacttgagcatatacaatgaatgtttcttaagatgtcaatatttgcttataatatagtgacttcccagtatatgtttcagttttgtttcttgcttagtgactagaacaaaaaaacaagtgttctattggtttaattaatctaaactgcattgctcaagcaataattgagtttattccctataacttgcaaagtgtggccatgttatgccctgtggctgtgcgtggccatctgacctccacatctatgtttcccactgctaggttgctttgagtcgtggtggatctcccggtgtgacgacatggggctgggtctgggagctcttctcaaatccgcgggctctcggtctgctcttctcaatttagtgttatctttttcttttagaacaatgccaaagaaacatgacagactgctttgcttgtttttgacatgatgcaaaagcaatggagtctttacttttaaacctttgtatttttgttttgattcaattctgatactgctgaaatgtacgaatatctattattttgatgcaatagtggtgttttgcgatgtttaacagcttgtgtaatccaattattaaccctgctttgtatagaagagtttcttcagaatatatcaattcatgtattctcattatggatattatgtggatattttctatctatgaatggcccctgcactttgaatcgcttatgtcattgttagcaatcacataatatttttcttttctcttagatttaatttgtataatcatataatcattcatatattgttacaacaggatttggttcagcttctcactttgttttaattctgatactgctggttctcttcttgccaggtgcgtgcggccacccggccgtggaccaagcgccgccgctgctcttcttgccaggtgcgtgcgtctcttcagctggccaaaatcaatcatcccaatgcttgtttctgaagggcagcatgtagctcgaggtgctggtcaaacggaggaatcattctggtttggtttctcttttgtttttgtacatagatgacgacgacgtgtctcccgatgcctccccgtcactggcacaccttggcatcgatcctcgaatctctacccccacacccacatctccccgctgccgaaccagccccgatttgccaccatggacgtcgatgacgtatcacccaatgtctccctgtctctgg

SEQ ID NO: 9 - DNA, 3132 bp, Zea mays
actgaaggcgggaaacgacaatctggcgcgcctgcctgcaggcatcgttgaagatgcctctgccgacagtggtcccaaagatggacccccacccacgaggagcatcgtggaaaaagaagacgttccaaccacgtcttcaaagcaagtggattgatgtgatatctccactgacgtaagggatgacgcacaatcccactatccttcgaggcctcatcgttgaagatgcctctgccgacagtggtcccaaagatggacccccacccacgaggagcatcgtggaaaaagaagacgttccaaccacgtcttcaaagcaagtggattgatgtgatatctccactgacgtaagggatgacgcacaatcccactatccttcgaagcttactcgaggtcattcatatgcttgagaagagagtcgggatagtccaaaataaaacaaaggtaagattacctggtcaaaagtgaaaacatcagttaaaaggtggtataaagtaaaatatcggtaataaaaggtggcccaaagtgaaatttactcttttctactattataaaaattgaggatgtttttgtcggtactttgatacgtcatttttgtatgaattggtttttaagtttattcgcttttggaaatgcatatctgtatttgagtcgggttttaagttcgtttgcttttgtaaatacagagggatttgtataagaaatatctttagaaaaacccatatgctaatttgacataatttttgagaaaaatatatattcaggcgaattctcacaatgaacaataataagattaaaatagctttcccccgttgcagcgcatgggtattttttctagtaaaaataaaagataaacttagactcaaaacatttacaaaaacaacccctaaagttcctaaagcccaaagtgctatccacgatccatagcaagcccagcccaacccaacccaacccaacccaccccagtccagccaactggacaatagtctccacacccccccactatcaccgtgagttgtccgcacgcaccgcacgtctcgcagccaaaaaaaaaaagaaagaaaaaaaagaaaaagaaaaaacagcaggtgggtccgggtcgtgggggccggaaacgcgaggaggatcgcgagccagcgacgaggccggccctccctccgcttccaaagaaacgccccccatcgccactatatacatacccccccctctcctcccatccccccaacccttctagaaccatcttccacacactcaagccacactattggagaacacacagggacaacacaccataagatccaagggaggcctccgccgccgccggtaaccaccccgcccctctcctctttctttctccgtttttttttccgtctcggtctcgatctttggccttggtagtttgggtgggcgagaggcggcttcgtgcgcgcccagatcggtgcgcgggaggggcgggatctcgcggctggggctctcgccggcgtggatccggcccggatctcgcggggaatggggctctcggatgtagatctgcgatccgccgttgttgggggagatgatggggggtttaaaatttccgccgtgctaaacaagatcaggaagaggggaaaagggcactatggtttatatttttatatatttctgctgcttcgtcaggcttagatgtgctagatctttctttcttctttttgtgggtagaatttgaatccctcagcattgttcatcggtagtttttcttttcatgatttgtgacaaatgcagcctcgtgcggagcttttttgtaggtagaagcggaccggtaccatgataaaactactatttacgtacatatgcacatacacatataaactatatgctctatatcatatggattacgcatgcgtgtgtatgtataaatataaaggcatcgtcacgcttcaagtttgtctcttttatattaaactgagagttttcctctcaaactttaccttttcttcttcgatcctagctcttaagaaccctaataattcattgatcaaaataatggcgattttgccggaaaactcttcaaacttggatcttactatctccgttccaggcttctcttcatcccctctctccgatgaaggaagtggcggaggaagagaccagctaaggctagacatgaatcggttaccgtcgtctgaagacggagacgatgaagaattcagtcacgatgatggctctgctcctccgcgaaagaaactccgtctaaccagagaacagtcacgtcttcttgaagatagtttcagacagaatcatacccttaatcccaaacaaaaggaagtacttgccaagcatttgatgctacggccaagacaaattgaagtttggtttcaaaaccgtagagcaaggagcaaattgaagcaaaccgagatggaatgcgagtatctcaaaaggtggtttggttcattaacggaagaaaaccacaggctccatagagaagtagaagagcttagagccataaaggttggcccaacaacggtgaactctgcctcgagccttactatgtgtcctcgctgcgagcgagttacccctgccgcgagcccttcgagggcggtggtgccggttccggctaagaaaacgtttccgccgcaagagcgtgatcgttgagtcggggcccgggctgcatgcgtttggacgtatgctcattcaggttggagccaatttggttgatgtgtgtgcgagttcttgcgagtctgatgagacatctctgtattgtgtttctttccccagtgttttctgtacttgtgtaatcggctaatcgccaacagattcggcgatgaataaatgagaaataaattgttctgattttgagtgcaaaaaaaaaggaattaagcttactcgagatccactagtgattaagcggccgcatcgatcgtgaagtttctcatctaagcccccatttggacgtgaatgtagacacgtcgaaataaagatttccgaattagaataatttgtttattgctttcgcctataaatacgacggatcgtaatttgtcgttttatcaaaatgtactttcattttataataacgctgcggacatctacatttttgaattgaaaaaaaattggtaattactctttctttttctccatattgaccatcatactcattgc

SEQ ID NO: 10 - DNA, 5744 bp, Zea mays
ctactattttggaacagagggaatagtaggtagtaatgtttcacaataaatcacagtgctaaaatgagatatgaccttagatcccatagctcattgcataaaagtacttgatcagttggtcactgtctttcagaaaaaccgcagtttaattaaacttaatggctgctggatcagatgctagatagcactatatcttaattcgttttgcatgaacaccttataatacagaaccttttcttttcttccagcaactagactctgcatcccttgtggaaatgtgaaccttggttcgtacatgacaaataatacaacatatcatgctacctatgcaacactgacttgatttcaatccttggtttacttgccacatcatacttatggtatatttgggtgaaaagtagatgtttcaagcagtttgtaaatcctaaatacatcatggtttactctggtgctacaactactgttttaaggagaaactattagctttgggatcatctagaatattagcatagcatcaacttcaggcacaactacaagagcagcacttgaaggggtaaaattcagtgctacctacgtaaatcataaaaaaaattatttgtttgaattcaagtgttttgggggttcaacaatgattctatgtagctataaatttttttgttgatttcatgtcatattgattattggtttgatttcacctgttttcttattgtcagccagaaccagcttactatttcggatgttgcaaggaaggcattccttcacagtgtatgtgatagttctctttatacatgtaagacagtgtacaagggcaaaactttgtatgaaattactctgtactgtttacaatgattacagggcatacttgtagtgtttgaggagcaagagacaaaactctacattttagatatataaagcaatagttctttaactcaaaccaaaatctggattagtcttgagcactttctaataatcatataatgctcatgtacctcaataactgcttcagttaatcacatcttttagtttagcactatgctatgatagtttacaaagtgcattgttagcttattttccccataggttctttaatcatatctattgtgctagattttactctgtcccattaggagacaaacaagttcgttcaatagcatatgacacttgtatgctggtaaaatgattgaatattttgtttgacacctattgtttgaaggatgtaagcaatctcatgtacctgttgttgctcgcaaggttcatccctcacaagtacaagatcaaagactcgaaagcttaggtatgaacccataaaactgaatacttaatatgggcacacagtgatgtttttactgaaggcgggaaacgacaatctggcgcgcctgcctgcaggcatcgttgaagatgcctctgccgacagtggtcccaaagatggacccccacccacgaggagcatcgtggaaaaagaagacgttccaaccacgtcttcaaagcaagtggattgatgtgatatctccactgacgtaagggatgacgcacaatcccactatccttcgaggcctcatcgttgaagatgcctctgccgacagtggtcccaaagatggacccccacccacgaggagcatcgtggaaaaagaagacgttccaaccacgtcttcaaagcaagtggattgatgtgatatctccactgacgtaagggatgacgcacaatcccactatccttcgaagcttactcgaggtcattcatatgcttgagaagagagtcgggatagtccaaaataaaacaaaggtaagattacctggtcaaaagtgaaaacatcagttaaaaggtggtataaagtaaaatatcggtaataaaaggtggcccaaagtgaaatttactcttttctactattataaaaattgaggatgtttttgtcggtactttgatacgtcatttttgtatgaattggtttttaagtttattcgcttttggaaatgcatatctgtatttgagtcgggttttaagttcgtttgcttttgtaaatacagagggatttgtataagaaatatctttagaaaaacccatatgctaatttgacataatttttgagaaaaatatatattcaggcgaattctcacaatgaacaataataagattaaaatagctttcccccgttgcagcgcatgggtattttttctagtaaaaataaaagataaacttagactcaaaacatttacaaaaacaacccctaaagttcctaaagcccaaagtgctatccacgatccatagcaagcccagcccaacccaacccaacccaacccaccccagtccagccaactggacaatagtctccacacccccccactatcaccgtgagttgtccgcacgcaccgcacgtctcgcagccaaaaaaaaaaagaaagaaaaaaaagaaaaagaaaaaacagcaggtgggtccgggtcgtgggggccggaaacgcgaggaggatcgcgagccagcgacgaggccggccctccctccgcttccaaagaaacgccccccatcgccactatatacatacccccccctctcctcccatccccccaacccttctagaaccatcttccacacactcaagccacactattggagaacacacagggacaacacaccataagatccaagggaggcctccgccgccgccggtaaccaccccgcccctctcctctttctttctccgtttttttttccgtctcggtctcgatctttggccttggtagtttgggtgggcgagaggcggcttcgtgcgcgcccagatcggtgcgcgggaggggcgggatctcgcggctggggctctcgccggcgtggatccggcccggatctcgcggggaatggggctctcggatgtagatctgcgatccgccgttgttgggggagatgatggggggtttaaaatttccgccgtgctaaacaagatcaggaagaggggaaaagggcactatggtttatatttttatatatttctgctgcttcgtcaggcttagatgtgctagatctttctttcttctttttgtgggtagaatttgaatccctcagcattgttcatcggtagtttttcttttcatgatttgtgacaaatgcagcctcgtgcggagcttttttgtaggtagaagcggaccggtaccatgataaaactactatttacgtacatatgcacatacacatataaactatatgctctatatcatatggattacgcatgcgtgtgtatgtataaatataaaggcatcgtcacgcttcaagtttgtctcttttatattaaactgagagttttcctctcaaactttaccttttcttcttcgatcctagctcttaagaaccctaataattcattgatcaaaataatggcgattttgccggaaaactcttcaaacttggatcttactatctccgttccaggcttctcttcatcccctctctccgatgaaggaagtggcggaggaagagaccagctaaggctagacatgaatcggttaccgtcgtctgaagacggagacgatgaagaattcagtcacgatgatggctctgctcctccgcgaaagaaactccgtctaaccagagaacagtcacgtcttcttgaagatagtttcagacagaatcatacccttaatcccaaacaaaaggaagtacttgccaagcatttgatgctacggccaagacaaattgaagtttggtttcaaaaccgtagagcaaggagcaaattgaagcaaaccgagatggaatgcgagtatctcaaaaggtggtttggttcattaacggaagaaaaccacaggctccatagagaagtagaagagcttagagccataaaggttggcccaacaacggtgaactctgcctcgagccttactatgtgtcctcgctgcgagcgagttacccctgccgcgagcccttcgagggcggtggtgccggttccggctaagaaaacgtttccgccgcaagagcgtgatcgttgagtcggggcccgggctgcatgcgtttggacgtatgctcattcaggttggagccaatttggttgatgtgtgtgcgagttcttgcgagtctgatgagacatctctgtattgtgtttctttccccagtgttttctgtacttgtgtaatcggctaatcgccaacagattcggcgatgaataaatgagaaataaattgttctgattttgagtgcaaaaaaaaaggaattaagcttactcgagatccactagtgattaagcggccgcatcgatcgtgaagtttctcatctaagcccccatttggacgtgaatgtagacacgtcgaaataaagatttccgaattagaataatttgtttattgctttcgcctataaatacgacggatcgtaatttgtcgttttatcaaaatgtactttcattttataataacgctgcggacatctacatttttgaattgaaaaaaaattggtaattactctttctttttctccatattgaccatcatactcattgcgatccacatttccctacatggtggaggatacagagcactcattccggagtataatcttgtcttgtgttgccacctatttatcacttgagcatatacaatgaatgtttcttaagatgtcaatatttgcttataatatagtgacttcccagtatatgtttcagttttgtttcttgcttagtgactagaacaaaaaaacaagtgttctattggtttaattaatctaaactgcattgctcaagcaataattgagtttattccctataacttgcaaagtgtggccatgttatgccctgtggctgtgcgtggccatctgacctccacatctatgtttcccactgctaggttgctttgagtcgtggtggatctcccggtgtgacgacatggggctgggtctgggagctcttctcaaatccgcgggctctcggtctgctcttctcaatttagtgttatctttttcttttagaacaatgccaaagaaacatgacagactgctttgcttgtttttgacatgatgcaaaagcaatggagtctttacttttaaacctttgtatttttgttttgattcaattctgatactgctgaaatgtacgaatatctattattttgatgcaatagtggtgttttgcgatgtttaacagcttgtgtaatccaattattaaccctgctttgtatagaagagtttcttcagaatatatcaattcatgtattctcattatggatattatgtggatattttctatctatgaatggcccctgcactttgaatcgcttatgtcattgttagcaatcacataatatttttcttttctcttagatttaatttgtataatcatataatcattcatatattgttacaacaggatttggttcagcttctcactttgttttaattctgatactgctggttctcttcttgccaggtgcgtgcggccacccggccgtggaccaagcgccgccgctgctcttcttgccaggtgcgtgcgtctcttcagctggccaaaatcaatcatcccaatgcttgtttctgaagggcagcatgtagctcgaggtgctggtcaaacggaggaatcattctggtttggtttctcttttgtttttgtacatagatgacgacgacgtgtctcccgatgcctccccgtcactggcacaccttggcatcgatcctcgaatctctacccccacacccacatctccccgctgccgaaccagccccgatttgccaccatggacgtcgatgacgtatcacccaatgtctccctgtctctgg

SEQ ID NO: 11 - DNA, 22 bp, Artificial sequence
  Primer
tgctctgtatcctccaccatgt

SEQ ID NO: 12 - DNA, 27 bp, Artificial sequence
  Primer
tttctccatattgaccatcatactcat

SEQ ID NO: 13 - DNA, 15 bp, Artificial sequence
  Primer
ctgatccacatttcc

SEQ ID NO: 14 - DNA, 27 bp, Artificial sequence
  Primer
gcatgtctttaaaaatccttggtttac

SEQ ID NO: 15 - DNA, 26 bp, Artificial sequence
  Primer
tgatgtttttactggattgcattacc

SEQ ID NO: 16 - DNA, 23 bp, Artificial sequence
  Primer
caccctaagagtactattgaaga

SEQ ID NO: 17 - DNA, 27 bp, Artificial sequence
  Primer
ttgttgctcgcaaggttcatccctcac

SEQ ID NO: 18 - DNA, 30 bp, Artificial sequence
  Primer
gacatcttaagaaacattcattgtatatgc

SEQ ID NO: 19 - DNA, 24 bp, Artificial sequence
  Primer
cccatttggacgtgaatgtagaca

SEQ ID NO: 20 - DNA, 24 bp, Artificial sequence
  Primer
ggacgtgaatgtagacacgtcgaa

SEQ ID NO: 21 - DNA, 24 bp, Artificial sequence
  Primer
tcgcctataaatacgacggatcgt

SEQ ID NO: 22 - DNA, 22 bp, Artificial sequence
  Primer
ctccaacctgaatgagcatacg

SEQ ID NO: 23 - DNA, 21 bp, Artificial sequence
  Primer
ctcgcaagaactcgcacacac

SEQ ID NO: 24 - DNA, 23 bp, Artificial sequence
  Primer
ggactatcccgactctcttctca

SEQ ID NO: 25 - DNA, 24 bp, Artificial sequence
  Primer
cacacagggacaacacaccataag

SEQ ID NO: 26 - DNA, 23 bp, Artificial sequence
  Primer
gcagaggcatcttcaacgatgag

SEQ ID NO: 27 - DNA, 25 bp, Artificial sequence
  Primer
ggacaacacaccataagatccaagg

SEQ ID NO: 28 - DNA, 21 bp, Artificial sequence
  Primer
aggcatcttcaacgatgaggc

SEQ ID NO: 29 - DNA, 21 bp, Artificial sequence
  Primer
gtagtttgggtgggcgagagg